European Patent Application EP 4 190 819 A1, published June 7, 2023. Title: PHARMACEUTICAL COMBINATION CONTAINING ANTI-PD-1-ANTI-VEGFA BISPECIFIC ANTIBODY, AND USE THEREOF. Applicant: Akeso Biopharma, Inc. The sequence listing filed with the application follows.

SEQUENCE LISTING (42 sequences)

SEQ ID NO: 1 - protein, 123 aa, Artificial Sequence [sequence omitted]

SEQ ID NO: 2 - DNA, 369 bp, Artificial Sequence
  nucleic acid encoding Bevacizumab-Hv
gaggtgcagctggtcgagtccgggggggggctggtgcagccaggcgggtctctgaggctgagttgcgccgcttcagggtacaccttcacaaactatggaatgaattgggtgcgccaggcaccaggaaagggactggagtgggtcggctggatcaacacttacaccggggaacctacctatgcagccgactttaagcggcggttcaccttcagcctggatacaagcaaatccactgcctacctgcagatgaacagcctgcgagctgaggacaccgcagtctactattgtgctaaatatccccactactatgggagcagccattggtattttgacgtgtgggggcaggggactctggtgacagtgagcagc

SEQ ID NO: 3 - protein, 107 aa, Artificial Sequence [sequence omitted]

SEQ ID NO: 4 - DNA, 321 bp, Artificial Sequence
  nucleic acid encoding Bevacizumab-Lv
gatattcagatgactcagagcccctcctccctgtccgcctctgtgggcgacagggtcaccatcacatgcagtgcttcacaggatatttccaactacctgaattggtatcagcagaagccaggaaaagcacccaaggtgctgatctacttcactagctccctgcactcaggagtgccaagccggttcagcggatccggatctggaaccgactttactctgaccatttctagtctgcagcctgaggatttcgctacatactattgccagcagtattctaccgtgccatggacatttggccaggggactaaagtcgagatcaag

SEQ ID NO: 5 - protein, 118 aa, Artificial Sequence
  VH of 14C12
EVKLVESGGGLVKPGGSLKLSCAASGFAFSSYDMSWVRQTPEKRLEWVATISGGGRYTYYPDSVKGRFTISRDNARNTLYLQMSSLRSEDTALYYCANRYGEAWFAYWGQGTLVTVSA

SEQ ID NO: 6 - DNA, 354 bp, Artificial Sequence
  nucleic acid encoding VH of 14C12
gaggtcaaactggtggagagcggcggcgggctggtgaagcccggcgggtcactgaaactgagctgcgccgcttccggcttcgcctttagctcctacgacatgtcatgggtgaggcagacccctgagaagcgcctggaatgggtcgctactatcagcggaggcgggcgatacacctactatcctgactctgtcaaagggagattcacaattagtcgggataacgccagaaatactctgtatctgcagatgtctagtctgcggtccgaggatacagctctgtactattgtgcaaaccggtacggcgaagcatggtttgcctattggggacagggcaccctggtgacagtctctgcc

SEQ ID NO: 7 - protein, 107 aa, Artificial Sequence
  VL of 14C12
DIKMTQSPSSMYASLGERVTFTCKASQDINTYLSWFQQKPGKSPKTLIYRANRLVDGVPSRFSGSGSGQDYSLTISSLEYEDMGIYYCLQYDEFPLTFGAGTKLELK

SEQ ID NO: 8 - DNA, 321 bp, Artificial Sequence
  nucleic acid encoding VL of 14C12
gacattaagatgacacagtccccttcctcaatgtacgctagcctgggcgagcgagtgaccttcacatgcaaagcatcccaggacatcaacacatacctgtcttggtttcagcagaagccaggcaaaagccccaagaccctgatctaccgggccaatagactggtggacggggtccccagcagattctccggatctggcagtgggcaggattactccctgaccatcagctccctggagtatgaagacatgggcatctactattgcctgcagtatgatgagttccctctgacctttggagcaggcacaaaactggaactgaag

SEQ ID NO: 9 - protein, 118 aa, Artificial Sequence
  VH of 14C12H1L1
EVQLVESGGGLVQPGGSLRLSCAASGFAFSSYDMSWVRQAPGKGLDWVATISGGGRYTYYPDSVKGRFTISRDNSKNNLYLQMNSLRAEDTALYYCANRYGEAWFAYWGQGTLVTVSS

SEQ ID NO: 10 - DNA, 354 bp, Artificial Sequence
  nucleic acid encoding VH of 14C12H1L1
gaagtgcagctggtcgagtctgggggagggctggtgcagcccggcgggtcactgcgactgagctgcgcagcttccggattcgcctttagctcctacgacatgtcctgggtgcgacaggcaccaggaaagggactggattgggtcgctactatctcaggaggcgggagatacacctactatcctgacagcgtcaagggccggttcacaatctctagagataacagtaagaacaatctgtatctgcagatgaacagcctgagggctgaggacaccgcactgtactattgtgccaaccgctacggggaagcatggtttgcctattgggggcagggaaccctggtgacagtctctagt

SEQ ID NO: 11 - protein, 107 aa, Artificial Sequence
  VL of 14C12H1L1
DIQMTQSPSSMSASVGDRVTFTCRASQDINTYLSWFQQKPGKSPKTLIYRANRLVSGVPSRFSGSGSGQDYTLTISSLQPEDMATYYCLQYDEFPLTFGAGTKLELK

SEQ ID NO: 12 - DNA, 321 bp, Artificial Sequence
  nucleic acid encoding VL of 14C12H1L1
gacattcagatgactcagagcccctcctccatgtccgcctctgtgggcgacagggtcaccttcacatgccgcgctagtcaggatatcaacacctacctgagctggtttcagcagaagccagggaaaagccccaagacactgatctaccgggctaatagactggtgtctggagtcccaagtcggttcagtggctcagggagcggacaggactacactctgaccatcagctccctgcagcctgaggacatggcaacctactattgcctgcagtatgatgagttcccactgacctttggcgccgggacaaaactggagctgaag

SEQ ID NO: 13 - protein, 448 aa, Artificial Sequence
  heavy chain of 14C12H1L1
EVQLVESGGGLVQPGGSLRLSCAASGFAFSSYDMSWVRQAPGKGLDWVATISGGGRYTYYPDSVKGRFTISRDNSKNNLYLQMNSLRAEDTALYYCANRYGEAWFAYWGQGTLVTVSSASTKGPSVFPLAPSSKSTSGGTAALGCLVKDYFPEPVTVSWNSGALTSGVHTFPAVLQSSGLYSLSSVVTVPSSSLGTQTYICNVNHKPSNTKVDKKVEPKSCDKTHTCPPCPAPELLGGPSVFLFPPKPKDTLMISRTPEVTCVVVDVSHEDPEVKFNWYVDGVEVHNAKTKPREEQYNSTYRVVSVLTVLHQDWLNGKEYKCKVSNKALPAPIEKTISKAKGQPREPQVYTLPPSRDELTKNQVSLTCLVKGFYPSDIAVEWESNGQPENNYKTTPPVLDSDGSFFLYSKLTVDKSRWQQGNVFSCSVMHEALHNHYTQKSLSLSPGK

SEQ ID NO: 14 - DNA, 1344 bp, Artificial Sequence
  nucleic acid encoding heavy chain of 14C12H1L1
gaagtgcagctggtcgagtctgggggagggctggtgcagcccggcgggtcactgcgactgagctgcgcagcttccggattcgcctttagctcctacgacatgtcctgggtgcgacaggcaccaggaaagggactggattgggtcgctactatctcaggaggcgggagatacacctactatcctgacagcgtcaagggccggttcacaatctctagagataacagtaagaacaatctgtatctgcagatgaacagcctgagggctgaggacaccgcactgtactattgtgccaaccgctacggggaagcatggtttgcctattgggggcagggaaccctggtgacagtctctagtgccagcaccaaaggacctagcgtgtttcctctcgccccctcctccaaaagcaccagcggaggaaccgctgctctcggatgtctggtgaaggactacttccctgaacccgtcaccgtgagctggaatagcggcgctctgacaagcggagtccatacattccctgctgtgctgcaaagcagcggactctattccctgtccagcgtcgtcacagtgcccagcagcagcctgggcacccagacctacatctgtaacgtcaaccacaagccctccaacaccaaggtggacaagaaagtggagcccaaatcctgcgacaagacacacacctgtcccccctgtcctgctcccgaactcctcggaggccctagcgtcttcctctttcctcccaaacccaaggacaccctcatgatcagcagaacccctgaagtcacctgtgtcgtcgtggatgtcagccatgaggaccccgaggtgaaattcaactggtatgtcgatggcgtcgaggtgcacaacgccaaaaccaagcccagggaggaacagtacaactccacctacagggtggtgtccgtgctgacagtcctccaccaggactggctgaacggcaaggagtacaagtgcaaggtgtccaacaaggctctccctgcccccattgagaagaccatcagcaaggccaaaggccaacccagggagccccaggtctatacactgcctccctccagggacgaactcaccaagaaccaggtgtccctgacctgcctggtcaagggcttttatcccagcgacatcgccgtcgagtgggagtccaacggacagcccgagaataactacaagaccacccctcctgtcctcgactccgacggctccttcttcctgtacagcaagctgaccgtggacaaaagcaggtggcagcagggaaacgtgttctcctgcagcgtgatgcacgaagccctccacaaccactacacccagaaaagcctgtccctgagccccggcaaa

SEQ ID NO: 15 - protein, 214 aa, Artificial Sequence
  light chain of 14C12H1L1
DIQMTQSPSSMSASVGDRVTFTCRASQDINTYLSWFQQKPGKSPKTLIYRANRLVSGVPSRFSGSGSGQDYTLTISSLQPEDMATYYCLQYDEFPLTFGAGTKLELKRTVAAPSVFIFPPSDEQLKSGTASVVCLLNNFYPREAKVQWKVDNALQSGNSQESVTEQDSKDSTYSLSSTLTLSKADYEKHKVYACEVTHQGLSSPVTKSFNRGEC

SEQ ID NO: 16 - DNA, 642 bp, Artificial Sequence
  lnucleic acid encoding ight chain of 14C12H1L1
gacattcagatgactcagagcccctcctccatgtccgcctctgtgggcgacagggtcaccttcacatgccgcgctagtcaggatatcaacacctacctgagctggtttcagcagaagccagggaaaagccccaagacactgatctaccgggctaatagactggtgtctggagtcccaagtcggttcagtggctcagggagcggacaggactacactctgaccatcagctccctgcagcctgaggacatggcaacctactattgcctgcagtatgatgagttcccactgacctttggcgccgggacaaaactggagctgaagcgaactgtggccgctccctccgtcttcatttttcccccttctgacgaacagctgaaatcaggcacagccagcgtggtctgtctgctgaacaatttctaccctagagaggcaaaagtgcagtggaaggtcgataacgccctgcagtccggcaacagccaggagagtgtgactgaacaggactcaaaagatagcacctattccctgtctagtacactgactctgtccaaggctgattacgagaagcacaaagtgtatgcatgcgaagtgacacatcagggactgtcaagccccgtgactaagtcttttaaccggggcgaatgt

SEQ ID NO: 17 - protein, 108 aa, Artificial Sequence
  light chain of 14C12H1L1(M)1
DIQMTQSPSSMSASVGDRVTFTCRASQDINTYLSWFQQKPGKSPKTLIYRANRLVSGVPSRFSGSGSGQDYTLTISSLQPEDMATYYCLQYDEFPLTFGAGTKLELKR

SEQ ID NO: 18 - protein, 20 aa, Artificial Sequence
  Linker 1
GGGGSGGGGSGGGGSGGGGS

SEQ ID NO: 19 - protein, 15 aa, Artificial Sequence
  linker 2
GGGGSGGGGSGGGGS

SEQ ID NO: 20 - protein, 453 aa, Artificial Sequence
  Bevacizumab-G4H
EVQLVESGGGLVQPGGSLRLSCAASGYTFTNYGMNWVRQAPGKGLEWVGWINTYTGEPTYAADFKRRFTFSLDTSKSTAYLQMNSLRAEDTAVYYCAKYPHYYGSSHWYFDVWGQGTLVTVSSASTKGPSVFPLAPSSKSTSGGTAALGCLVKDYFPEPVTVSWNSGALTSGVHTFPAVLQSSGLYSLSSVVTVPSSSLGTQTYICNVNHKPSNTKVDKKVEPKSCDKTHTCPPCPAPELLGGPSVFLFPPKPKDTLMISRTPEVTCVVVDVSHEDPEVKFNWYVDGVEVHNAKTKPREEQYNSTYRVVSVLTVLHQDWLNGKEYKCKVSNKALPAPIEKTISKAKGQPREPQVYTLPPSRDELTKNQVSLTCLVKGFYPSDIAVEWESNGQPENNYKTTPPVLDSDGSFFLYSKLTVDKSRWQQGNVFSCSVMHEALHNHYTQKSLSLSPGK

SEQ ID NO: 21 - DNA, 1359 bp, Artificial Sequence
  nucleic acid encoding Bevacizumab-G4H
gaggtgcagctggtcgagtccgggggggggctggtgcagccaggcgggtctctgaggctgagttgcgccgcttcagggtacaccttcacaaactatggaatgaattgggtgcgccaggcaccaggaaagggactggagtgggtcggctggatcaacacttacaccggggaacctacctatgcagccgactttaagcggcggttcaccttcagcctggatacaagcaaatccactgcctacctgcagatgaacagcctgcgagctgaggacaccgcagtctactattgtgctaaatatccccactactatgggagcagccattggtattttgacgtgtgggggcaggggactctggtgacagtgagcagcgcaagcaccaaagggcccagcgtgtttcctctcgccccctcctccaaaagcaccagcggaggaaccgctgctctcggatgtctggtgaaggactacttccctgaacccgtcaccgtgagctggaatagcggcgctctgacaagcggagtccatacattccctgctgtgctgcaaagcagcggactctattccctgtccagcgtcgtcacagtgcccagcagcagcctgggcacccagacctacatctgtaacgtcaaccacaagccctccaacaccaaggtggacaagaaagtggagcccaaatcctgcgacaagacacacacctgtcccccctgtcctgctcccgaactcctcggaggccctagcgtcttcctctttcctcccaaacccaaggacaccctcatgatcagcagaacccctgaagtcacctgtgtcgtcgtggatgtcagccatgaggaccccgaggtgaaattcaactggtatgtcgatggcgtcgaggtgcacaacgccaaaaccaagcccagggaggaacagtacaactccacctacagggtggtgtccgtgctgacagtcctccaccaggactggctgaacggcaaggagtacaagtgcaaggtgtccaacaaggctctccctgcccccattgagaagaccatcagcaaggccaaaggccaacccagggagccccaggtctatacactgcctccctccagggacgaactcaccaagaaccaggtgtccctgacctgcctggtcaagggcttttatcccagcgacatcgccgtcgagtgggagtccaacggacagcccgagaataactacaagaccacccctcctgtcctcgactccgacggctccttcttcctgtacagcaaactgaccgtcgataaatctaggtggcagcagggcaacgtgttctcttgttccgtgatgcatgaagcactgcacaaccattatacccagaagtctctgagcctgtcccccggcaag

SEQ ID NO: 22 - protein, 450 aa, Artificial Sequence
  heavy chain of VP101(hG4WT)
EVQLVESGGGLVQPGGSLRLSCAASGYTFTNYGMNWVRQAPGKGLEWVGWINTYTGEPTYAADFKRRFTFSLDTSKSTAYLQMNSLRAEDTAVYYCAKYPHYYGSSHWYFDVWGQGTLVTVSSASTKGPSVFPLAPCSRSTSESTAALGCLVKDYFPEPVTVSWNSGALTSGVHTFPAVLQSSGLYSLSSVVTVPSSSLGTKTYTCNVDHKPSNTKVDKRVESKYGPPCPPCPAPEFLGGPSVFLFPPKPKDTLMISRTPEVTCVVVDVSQEDPEVQFNWYVDGVEVHNAKTKPREEQFNSTYRVVSVLTVLHQDWLNGKEYKCKVSNKGLPSSIEKTISKAKGQPREPQVYTLPPSQEEMTKNQVSLTCLVKGFYPSDIAVEWESNGQPENNYKTTPPVLDSDGSFFLYSRLTVDKSRWQEGNVFSCSVMHEALHNHYTQKSLSLSLGK

SEQ ID NO: 23 - DNA, 1350 bp, Artificial Sequence
  nucleic acid encoding heavy chain of VP101(hG4WT)
gaggtgcagctggtcgagtccgggggggggctggtgcagccaggcgggtctctgaggctgagttgcgccgcttcagggtacaccttcacaaactatggaatgaattgggtgcgccaggcaccaggaaagggactggagtgggtcggctggatcaacacttacaccggggaacctacctatgcagccgactttaagcggcggttcaccttcagcctggatacaagcaaatccactgcctacctgcagatgaacagcctgcgagctgaggacaccgcagtctactattgtgctaaatatccccactactatgggagcagccattggtattttgacgtgtgggggcaggggactctggtgacagtgagcagcgcaagcaccaaagggccctcggtcttccccctggcgccctgctccaggagcacctccgagagcacagccgccctgggctgcctggtcaaggactacttccccgaaccggtgacggtgtcgtggaactcaggcgccctgaccagcggcgtgcacaccttcccggctgtcctacagtcctcaggactctactccctcagcagcgtggtgaccgtgccctccagcagcttgggcacgaagacctacacctgcaacgtagatcacaagcccagcaacaccaaggtggacaagagagttgagtccaaatatggtcccccatgcccaccatgcccagcacctgagttcctggggggaccatcagtcttcctgttccccccaaaacccaaggacactctcatgatctcccggacccctgaggtcacgtgcgtggtggtggacgtgagccaggaagaccccgaggtccagttcaactggtacgtggatggcgtggaggtgcataatgccaagacaaagccgcgggaggagcagttcaacagcacgtaccgtgtggtcagcgtcctcaccgtcctgcaccaggactggctgaacggcaaggagtacaagtgcaaggtctccaacaaaggcctcccgtcctccatcgagaaaaccatctccaaagccaaagggcagccccgagagccacaggtgtacaccctgcccccatcccaggaggagatgaccaagaaccaggtcagcctgacctgcctggtcaaaggcttctaccccagcgacatcgccgtggagtgggagagcaatgggcagccggagaacaactacaagaccacgcctcccgtgctggactccgacggctccttcttcctctacagcaggctaaccgtggacaagagcaggtggcaggaggggaatgtcttctcatgctccgtgatgcatgaggctctgcacaaccactacacacagaagtctctgagcctgtccctcggcaag

SEQ ID NO: 24 - protein, 453 aa, Artificial Sequence
  Immunoglobulin heavy  chain of VP101(hG1DM)
EVQLVESGGGLVQPGGSLRLSCAASGYTFTNYGMNWVRQAPGKGLEWVGWINTYTGEPTYAADFKRRFTFSLDTSKSTAYLQMNSLRAEDTAVYYCAKYPHYYGSSHWYFDVWGQGTLVTVSSASTKGPSVFPLAPSSKSTSGGTAALGCLVKDYFPEPVTVSWNSGALTSGVHTFPAVLQSSGLYSLSSVVTVPSSSLGTQTYICNVNHKPSNTKVDKKVEPKSCDKTHTCPPCPAPEAAGGPSVFLFPPKPKDTLMISRTPEVTCVVVDVSHEDPEVKFNWYVDGVEVHNAKTKPREEQYNSTYRVVSVLTVLHQDWLNGKEYKCKVSNKALPAPIEKTISKAKGQPREPQVYTLPPSRDELTKNQVSLTCLVKGFYPSDIAVEWESNGQPENNYKTTPPVLDSDGSFFLYSKLTVDKSRWQQGNVFSCSVMHEALHNHYTQKSLSLSPGK

SEQ ID NO: 25 - DNA, 1359 bp, Artificial Sequence
  nucleic acid encoding Immunoglobulin heavy  chain of VP101(hG1DM)
gaggtgcagctggtcgagtccgggggggggctggtgcagccaggcgggtctctgaggctgagttgcgccgcttcagggtacaccttcacaaactatggaatgaattgggtgcgccaggcaccaggaaagggactggagtgggtcggctggatcaacacttacaccggggaacctacctatgcagccgactttaagcggcggttcaccttcagcctggatacaagcaaatccactgcctacctgcagatgaacagcctgcgagctgaggacaccgcagtctactattgtgctaaatatccccactactatgggagcagccattggtattttgacgtgtgggggcaggggactctggtgacagtgagcagcgcaagcaccaaagggcccagcgtgtttcctctcgccccctcctccaaaagcaccagcggaggaaccgctgctctcggatgtctggtgaaggactacttccctgaacccgtcaccgtgagctggaatagcggcgctctgacaagcggagtccatacattccctgctgtgctgcaaagcagcggactctattccctgtccagcgtcgtcacagtgcccagcagcagcctgggcacccagacctacatctgtaacgtcaaccacaagccctccaacaccaaggtggacaagaaagtggagcccaaatcctgcgacaagacacacacctgtcccccctgtcctgctcccgaagctgctggaggccctagcgtcttcctctttcctcccaaacccaaggacaccctcatgatcagcagaacccctgaagtcacctgtgtcgtcgtggatgtcagccatgaggaccccgaggtgaaattcaactggtatgtcgatggcgtcgaggtgcacaacgccaaaaccaagcccagggaggaacagtacaactccacctacagggtggtgtccgtgctgacagtcctccaccaggactggctgaacggcaaggagtacaagtgcaaggtgtccaacaaggctctccctgcccccattgagaagaccatcagcaaggccaaaggccaacccagggagccccaggtctatacactgcctccctccagggacgaactcaccaagaaccaggtgtccctgacctgcctggtcaagggcttttatcccagcgacatcgccgtcgagtgggagtccaacggacagcccgagaataactacaagaccacccctcctgtcctcgactccgacggctccttcttcctgtacagcaaactgaccgtcgataaatctaggtggcagcagggcaacgtgttctcttgttccgtgatgcatgaagcactgcacaaccattatacccagaagtctctgagcctgtcccccggcaag

SEQ ID NO: 26 - protein, 214 aa, Artificial Sequence
  Immunoglobulin light chain of VP101(hG1DM)
DIQMTQSPSSLSASVGDRVTITCSASQDISNYLNWYQQKPGKAPKVLIYFTSSLHSGVPSRFSGSGSGTDFTLTISSLQPEDFATYYCQQYSTVPWTFGQGTKVEIKRTVAAPSVFIFPPSDEQLKSGTASVVCLLNNFYPREAKVQWKVDNALQSGNSQESVTEQDSKDSTYSLSSTLTLSKADYEKHKVYACEVTHQGLSSPVTKSFNRGEC

SEQ ID NO: 27 - DNA, 642 bp, Artificial Sequence
  nucleic acid encoding Immunoglobulin light chain of VP101(hG1DM)
gatattcagatgactcagagcccctcctccctgtccgcctctgtgggcgacagggtcaccatcacatgcagtgcttcacaggatatttccaactacctgaattggtatcagcagaagccaggaaaagcacccaaggtgctgatctacttcactagctccctgcactcaggagtgccaagccggttcagcggatccggatctggaaccgactttactctgaccatttctagtctgcagcctgaggatttcgctacatactattgccagcagtattctaccgtgccatggacatttggccaggggactaaagtcgagatcaagcggaccgtggccgctcccagtgtcttcatttttccccctagcgacgaacagctgaaatccgggacagcctctgtggtctgtctgctgaacaacttctaccctagagaggcaaaagtgcagtggaaggtcgataacgccctgcagagtggcaattcacaggagagcgtgacagaacaggactccaaagattctacttatagtctgtcaagcacactgactctgagcaaggctgactacgaaaagcataaagtgtatgcatgtgaggtcacccaccaggggctgagcagtccagtcaccaagtcattcaacagaggcgagtgc

SEQ ID NO: 28 - protein, 8 aa, Artificial Sequence
  HCDR1
GYTFTNYG

SEQ ID NO: 29 - protein, 8 aa, Artificial Sequence
  HCDR2
INTYTGEP

SEQ ID NO: 30 - protein, 16 aa, Artificial Sequence
  HCDR3
AKYPHYYGSSHWYFDV

SEQ ID NO: 31 - protein, 6 aa, Artificial Sequence
  LCDR1
QDISNY

SEQ ID NO: 32 - protein, 3 aa, Artificial Sequence
  LCDR2
FTS

SEQ ID NO: 33 - protein, 9 aa, Artificial Sequence
  LCDR3
QQYSTVPWT

SEQ ID NO: 34 - protein, 8 aa, Artificial Sequence
  HCDR1
GFAFSSYD

SEQ ID NO: 35 - protein, 8 aa, Artificial Sequence
  HCDR2
ISGGGRYT

SEQ ID NO: 36 - protein, 11 aa, Artificial Sequence
  HCDR3
ANRYGEAWFAY

SEQ ID NO: 37 - protein, 6 aa, Artificial Sequence
  LCDR1
QDINTY

SEQ ID NO: 38 - protein, 3 aa, Artificial Sequence
  LCDR2
RAN

SEQ ID NO: 39 - protein, 9 aa, Artificial Sequence
  LCDR3
LQYDEFPLT

SEQ ID NO: 40 - protein, 330 aa, Artificial Sequence [sequence omitted]

SEQ ID NO: 41 - protein, 327 aa, Artificial Sequence
  Ig gamma-4 chain C region
ASTKGPSVFPLAPCSRSTSESTAALGCLVKDYFPEPVTVSWNSGALTSGVHTFPAVLQSSGLYSLSSVVTVPSSSLGTKTYTCNVDHKPSNTKVDKRVESKYGPPCPSCPAPEFLGGPSVFLFPPKPKDTLMISRTPEVTCVVVDVSQEDPEVQFNWYVDGVEVHNAKTKPREEQFNSTYRVVSVLTVLHQDWLNGKEYKCKVSNKGLPSSIEKTISKAKGQPREPQVYTLPPSQEEMTKNQVSLTCLVKGFYPSDIAVEWESNGQPENNYKTTPPVLDSDGSFFLYSRLTVDKSRWQEGNVFSCSVMHEALHNHYTQKSLSLSLGK

SEQ ID NO: 42 - protein, 107 aa, Artificial Sequence [sequence omitted]